European Patent Application EP 4 159 865 A1, published April 5, 2023. Title: E. COLI VARIANT STRAIN OR CORYNEBACTERIUM GLUTAMICUM VARIANT STRAIN PRODUCING L-AMINO ACIDS, AND METHOD FOR PRODUCING L-AMINO ACIDS USING SAME. Applicant: DAESANG CORPORATION. Application EP, filed August 10, 2022. The sequence listing filed with the application follows.

SEQUENCE LISTING (39 sequences)

SEQ ID NO: 1 - DNA, 924 bp, synthetic construct
  misc_feature 1..924: note = yicL
  source 1..924: mol_type = other DNA
atgggttccaccagaaaggggatgctgaacgttctgattgccgccgtgttgtggggaagttcaggggtctgcgcgcaatacatcatggagcaaagccagatgtcgtcgcagtttttgactatgacgcgtttgatattcgccggtttgattctactgacgctgtcatttgttcatggcgataaaatcttttctattattaacaatcataaagatgccattagcctgctgattttttccgtggttggcgcgctaactgtacagctcacttttttgctaaccatcgaaaaatcgaacgcagccacggcaacggtgctgcaattcctctcaccgacgattatcgtcgcctggttctcactggtgcgtaaatcgcgcccgggcattctggttttctgcgctattttgacatcgctggtcgggacttttttattggtgacacacggtaatccgacgtcattatcgatctctcctgccgcgttgttctggggcattgcctcggcatttgctgctgcattctataccacctatccctcaacgctaattgcccgctatggcacgttaccagtcgtcggctggagtatgctgattggcggtctgattctgttgcctttttatgccagacaaggaacaaactttgtcgttaacggcagtttgattctggcgtttttttatttggtggtcattggtacgtccctgacatttagtctgtacctgaaaggagcacaattaattggcggtccaaaagccagcattttgagctgtgcagaaccattaagtagcgcgctactctctttgctgttgctggggatcacgttcacattaccggactggctgggaacgctgctgattctgtcatcggtgattttgatttcaatggattcccgtcgccgcgccagaaaaataaatcgtccggcgcggcataagtga

SEQ ID NO: 2 - DNA, 1266 bp, synthetic construct
  misc_feature 1..1266: note = ydiN
  source 1..1266: mol_type = other DNA
atgtctcaaaataaggctttcagcacgccatttatcctggctgttctttgtatttacttcagctacttcctgcacggcattagtgttattacgcttgcccaaaatatgtcatctctggcggaaaagttttccactgacaacgcgggcattgcctacttaatttccggtatcggtttggggcgattgatcagtattttattcttcggtgtgatctccgataagtttggtcgtcgggcggtgatattaatggcagtaataatgtatctgctattcttctttggtattcccgcttgcccgaatttaactctcgcctacggtctggcagtgtgcgtaggtatcgctaactcagcgctggatacgggtggctaccccgcgctcatggaatgctttccgaaagcctctggttcggcggtcatactggttaaagcgatggtgtcatttgggcaaatgttctacccaatgctggtgagctatatgttgctcaataatatctggtacggctatgggctgattattccgggtattctatttgtactgatcacgctgatgctgttgaaaagcaaattccccagccagttggtggacgccagcgtaactaatgaattaccgcaaatgaacagcaaaccgttagtctggctggaaggtgtttcatcggtactgttcggtgtagccgcattctcgaccttttatgtgattgtggtgtggatgcccaaatatgcgatggcttttgctggtatgtcagaagctgaggcattaaaaaccatctcttattacagtatgggctcgttggtctgtgtctttatttttgccgcactactgaaaaaaatggtccggcccatctgggctaatgtatttaactctgcactggcaacaataacagcagccattatctacctgtacccttctccactggtgtgcaatgccggagcctttgttatcggtttctcagcagctggcggcattttacagctcggcgtttcggtcatgtcagagttttttcccaaaagcaaagccaaagtcaccagtatttatatgatgatgggtggactggctaactttgttattccactgattaccggttatctgtcgaacatcggcctgcaatatatcattgttctcgattttactttcgcgctgctggccctgattaccgcaattattgtttttatccgctattaccgcgttttcattattcctgaaaatgatgtgcggtttggcgagcgtaaattttgcacccggttaaacacaattaagcatagaggttaa

SEQ ID NO: 3 - DNA, 2013 bp, synthetic construct
  misc_feature 1..2013: note = ydhK
  source 1..2013: mol_type = other DNA
atgaacgcatcgtcatggtccttgcgcaatttgccctggttcagggccacgctggcgcaatggcgttatgcgttacgcaataccattgccatgtgtctggcgctgacggttgcctattatttaaatctggatgaaccctattgggcgatgacctcggctgcagtggttagctttcccaccgttggcggtgttatcagcaaaagcctcggacgcatcgctggcagtttgctcggagccattgcggcactgcttcttgccgggcatacgctcaatgagccgtggttttttctattgagcatgtcggcgtggcttggcttttgtacctgggcctgtgcgcacttcacgaataacgtcgcgtatgcatttcaactggcgggctacacggctgccatcatcgcctttccgatggttaatattactgaggccagccagctgtgggatatcgctcaggcgcgcgtttgcgaggtaatagtcggtattttgtgcggcggcatgatgatgatgatcctgccgagcagttccgatgctactgcccttttaaccgcattgaaaaacatgcacgcccgattactggaacatgccagtttactctggcagcctgaaacaaccgatgccattcgtgcagcacatgaaggggtgattgggcagatactgaccatgaatttgctgcgtatccaggctttctggagccactatcgttttcgccagcaaaacgcgcgccttaatgcgctgctccaccagcaattacgtatgaccagtgtcatctccagcctgcgacgtatgttgctcaactggccctcaccgccaggtgccacacgagaaattctcgaacagttgctgacggcgctcgccagttcgcaaacagatgtttacaccgtcgcacgtattatcgccccgctacgcccgaccaacgtcgccgactatcggcacgtcgccttctggcagcgactacgttatttttgccgcctttatctgcaaagtagtcaggaattacatcgtctgcaaagcggtgtagatgatcataccagactcccacggacatccggcctggctcgtcataccgataacgccgaagctatgtggagcgggctgcgtacattttgtacgttgatgatgattggcgcatggagtattgcttcgcaatgggatgccggtgccaatgcattaacgctggcagcaattagctgcgtactctactccgccgtcgcagcaccgtttaagtcgttgtcacttctgatgcgcacgctggtgttactttcgctattcagctttgtggtcaaatttggtctgatggtccagattagcgatctgtggcaatttttactgtttctctttccactgctggcgacaatgcagcttcttaaattgcagatgccaaaatttgccgcattgtgggggcaactgattgtttttatgggttcttttatcgctgtcactaatcccccggtgtatgattttgctgattttcttaacgataatctggcaaaaatcgttggcgtcgcgttggcgtggttagcgttcgccattctgcgtccaggatcggatgctcgtaaaagccgccgccatattcgcgcgctgcgccgggattttgtcgatcagctaagccgccatccaacactgagtgaaagcgaatttgaatcgctcacttatcatcacgtcagtcagttgagtaacagccaggatgcgctggctcgccgttggttattacgctggggtgtagtgctgctgaactgttctcatgttgtctggcaattgcgcgactgggaatcgcgttccgatccgttatcgcgagtacgggataactgtatttcactgttgcggggagtgatgagtgagcgtggcgttcagcaaaaatcactggcggccacacttgaagaattacagcggatttgcgacagccttgcccgtcatcatcaacctgccgcccgtgagctggcggcaattatctggcggctgtactgctcgctttcgcaacttgagcaagcaccaccgcaaggtacgctggcctcttaa

SEQ ID NO: 4 - DNA, 1968 bp, synthetic construct
  misc_feature 1..1968: note = aaeB
  source 1..1968: mol_type = other DNA
atgggtattttctccattgctaaccaacatattcgctttgcggtaaaactggcgaccgccattgtactggcgctgtttgttggctttcacttccagctggaaacgccacgctgggcggtactgacagcggcgattgttgccgccggtacggcctttgctgcgggaggtgaaccgtattctggcgctattcgctatcgtggctttttgcgcatcatcggcacatttattggctgtattgccggactggtgatcatcattgcgatgatccgcgcaccattattgatgattctggtgtgctgtatctgggccggtttttgtacctggatatcctcgctggtacgaatagaaaactcgtatgcgtgggggctggccggttataccgcgctgatcattgtgatcaccattcagccggaaccattgcttacgccgcagtttgccgtcgaacgttgtagcgagatcgttatcggtattgtgtgtgcgattatggcggatttgctcttttctccgcgatcgatcaaacaagaagtggatcgagagctggaaagtttgctggtcgcgcaatatcaattaatgcaactctgtatcaagcatggcgatggtgaagttgtcgataaagcctggggcgacctggtgcgacgcaccacggcgctacaaggcatgcgcagcaacctgaatatggaatcttcccgctgggcgcgggccaatcgacgtttaaaagcgatcaatacgctatcgctgacgctgattacccaatcctgcgaaacttatcttattcagaatacgcgcccggaattgatcactgatactttccgcgaattttttgacacgccggtagaaaccgcgcaggacgtccacaagcagctcaaacgcctgcggagagttatcgcctggaccggggaacgggaaacgcctgtcaccatttatagctgggtcgcggcggcaacgcgttatcagcttctcaagcgcggcgttatcagtaacacaaaaatcaacgccaccgaagaagagatcctgcaaggcgaaccggaagtaaaagtagagtcagccgaacgtcatcatgcaatggttaacttctggcgaaccacactttcctgcattctgggcacgcttttctggctgtggacgggctggacttccggcagtggtgcaatggtgatgattgcggtagtgacgtcactggcaatgcgtttgccgaatccacgcatggtggcgatcgactttatctacgggacgctggccgcgctgccgttagggctgctctactttttggtgattatccctaatacccaacagagcatgttgctgctgtgcattagcctggcagtgctgggattcttcctcggtatagaagtacagaaacggcgactgggctcgatgggggcactggccagcaccataaatattatcgtgctggataacccgatgactttccatttcagtcagtttctcgacagcgcattagggcaaatcgtcggctgtgtgctcgcgttcaccgttattttgctggtgcgggataaatcgcgcgacaggaccggacgtgtactgcttaatcagtttgtttctgccgctgtttccgcgatgactaccaatgtggcacgtcgtaaagagaaccacctcccggcactttatcagcagctgtttttgctgatgaataagttcccaggggatttgccgaaatttcgcctggcgctgacgatgattatcgcgcaccagcgcctgcgtgatgcaccgatcccggttaacgaggatttatcggcgtttcaccgacaaatgcgccgcacagcagaccatgtgatatctgcccgtagcgatgataaacgtcgtcggtactttggccagttgctggaagaactggaaatctaccaggaaaagctacgcatctggcaagcgccaccgcaggtgacggaaccggtaaatcggctggcggggatgctccataagtatcaacatgcgttgaccgatagttaa

SEQ ID NO: 5 - DNA, 1059 bp, synthetic construct
  misc_feature 1..1059: note = yeeA
  source 1..1059: mol_type = other DNA
gtgcgtgccgataagtcattaagcccgtttgaaatccgggtataccgccattaccgcattgtgcatggtactcgggtcgcgctggcattcctgctcacttttctcattatccgcctgtttactatcccggaaagcacctggccgctggtcaccatggtggtgattatggggccaatctcgttctggggtaacgttgtccctcgcgcctttgagcgtattggcggtacggtgttgggttcgattttaggtcttatcgctctgcaactggagttaatctcgttaccgctgatgttagtctggtgcgcggcggccatgttcctttgcggttggctggcgctgggcaagaaaccgtatcaaggtttattgattggggtgacgctggcaattgttgtgggttccccgacaggtgaaattgatacggcgttatggcgaagcggcgatgtgatcctcggctctttactggcaatgttgtttaccggtatctggccacaacgggcgttcatccactggcgcattcaactggcgaaaagtctgaccgagtataatcgggtctatcaatctgcattctcaccgaacttactcgaacgcccacgtctggaaagccatctacaaaaactcctgaccgatgccgtgaaaatgcgtggactgattgcgcccgccagcaaagaaacccgtattccaaaatcgatatatgaaggtatccagaccattaaccgcaatctggtttgtatgctggagttgcaaatcaatgcatactgggccacgcgccccagccatttcgtgttattgaacgcgcaaaaacttcgtgatacccagcacatgatgcagcaaatactgctgagccttgttcatgcgctgtacgaaggtaatccgcagccggtttttgccaatacggaaaaattgaacgatgctgtggaagagctgcgtcagttgctcaataaccaccatgacctgaaggttgtggaaacaccaatctatggttatgtgtggctgaacatggaaacggcgcatcagcttgagttgctatcgaatctgatttgccgggccttgcgcaaataa

SEQ ID NO: 6 - DNA, 621 bp, synthetic construct
  misc_feature 1..621: note = rhtC
  source 1..621: mol_type = other DNA
atgttgatgttatttctcaccgtcgccatggtgcacattgtggcgcttatgagccccggtcccgatttcttttttgtctctcagaccgctgtcagtcgttcccgtaaagaagcgatgatgggcgtgctgggcattacctgcggcgtaatggtttgggctgggattgcgctgcttggcctgcatttgattatcgaaaaaatggcctggctgcatacgctgattatggtgggcggtggcctgtatctctgctggatgggttaccagatgctacgtggtgcactgaaaaaagaggcggtttctgcacctgcgccacaggtcgagctggcgaaaagtgggcgcagtttcctgaaaggtttactgaccaatctcgctaatccgaaagcgattatctactttggctcggtgttctcattgtttgtcggtgataacgttggcactaccgcgcgctggggcatttttgcgctgatcattgtcgaaacgctggcgtggtttaccgtcgttgccagcctgtttgccctgccgcaaatgcgccgtggttatcaacgtctggcgaagtggattgatggttttgccggggcgttatttgccggatttggcattcatttgattatttcgcggtga

SEQ ID NO: 7 - DNA, 1185 bp, synthetic construct
  misc_feature 1..1185: note = emrD
  source 1..1185: mol_type = other DNA
atgaaaaggcaaagaaacgtcaatttgttattgatgttggtattactcgtggccgtcggtcagatggcgcaaaccatttatattccagctattgccgatatggcgcgcgatctcaacgtccgtgaaggggcggtgcagagcgtaatgggcgcttatctgctgacttacggtgtctcacagctgttttatggcccgatttccgaccgcgtgggccgccgaccggtgatcctcgtcggaatgtccatttttatgctggcaacgctggtcgcggtcacgacctccagtttgacggtgttgattgccgccagcgcgatgcaggggatgggcaccggcgttggcggcgtaatggcgcgtactttaccgcgagatttatatgaacggacacagttgcgccatgctaacagcctgttaaacatggggattctcgtcagtccgttgctcgcaccgctaatcggcggtctgctggatacgatgtggaactggcgcgcctgttatctctttttgttggttctttgtgctggtgtgaccttcagtatggcccgctggatgccggaaacgcgtccggtcgatgcaccgcgcacgcgcctgcttaccagttataaaacgcttttcggtaacagcggttttaactgttatttgctgatgctgattggcggtctggccgggattgccgcctttgaagcctgctccggcgtgctgatgggcgcggtgttagggctgagcagtatgacggtcagtattttgtttattctgccgattccggcagcgttttttggcgcatggtttgccggacgtcccaataaacgcttctccacgttaatgtggcagtcggttatctgctgcctgctggctggcttgctgatgtggatccccgactggtttggcgtgatgaatgtctggacgctgctcgttcccgccgcgctgttctttttcggtgccgggatgctgtttccgctggcgaccagcggcgcgatggagccgttccccttcctggcgggcacggctggcgcgctggtcggcggtctgcaaaacattggttccggcgtgctggcgtcgctctctgcgatgttaccgcaaaccggtcagggcagcctggggttgttgatgaccttaatgggattgttgatcgtgctgtgctggctgccgctggcgacgcggatgtcgcatcaggggcagcccgtttaa

SEQ ID NO: 8 - protein, 307 aa, synthetic construct
  REGION 1..307: note = yicL
MGSTRKGMLNVLIAAVLWGSSGVCAQYIMEQSQMSSQFLTMTRLIFAGLILLTLSFVHGDKIFSIINNHKDAISLLIFSVVGALTVQLTFLLTIEKSNAATATVLQFLSPTIIVAWFSLVRKSRPGILVFCAILTSLVGTFLLVTHGNPTSLSISPAALFWGIASAFAAAFYTTYPSTLIARYGTLPVVGWSMLIGGLILLPFYARQGTNFVVNGSLILAFFYLVVIGTSLTFSLYLKGAQLIGGPKASILSCAEPLSSALLSLLLLGITFTLPDWLGTLLILSSVILISMDSRRRARKINRPARHK

SEQ ID NO: 9 - protein, 421 aa, synthetic construct
  REGION 1..421: note = ydiN
MSQNKAFSTPFILAVLCIYFSYFLHGISVITLAQNMSSLAEKFSTDNAGIAYLISGIGLGRLISILFFGVISDKFGRRAVILMAVIMYLLFFFGIPACPNLTLAYGLAVCVGIANSALDTGGYPALMECFPKASGSAVILVKAMVSFGQMFYPMLVSYMLLNNIWYGYGLIIPGILFVLITLMLLKSKFPSQLVDASVTNELPQMNSKPLVWLEGVSSVLFGVAAFSTFYVIVVWMPKYAMAFAGMSEAEALKTISYYSMGSLVCVFIFAALLKKMVRPIWANVFNSALATITAAIIYLYPSPLVCNAGAFVIGFSAAGGILQLGVSVMSEFFPKSKAKVTSIYMMMGGLANFVIPLITGYLSNIGLQYIIVLDFTFALLALITAIIVFIRYYRVFIIPENDVRFGERKFCTRLNTIKHRG

SEQ ID NO: 10 - protein, 670 aa, synthetic construct
  REGION 1..670: note = ydhK
MNASSWSLRNLPWFRATLAQWRYALRNTIAMCLALTVAYYLNLDEPYWAMTSAAVVSFPTVGGVISKSLGRIAGSLLGAIAALLLAGHTLNEPWFFLLSMSAWLGFCTWACAHFTNNVAYAFQLAGYTAAIIAFPMVNITEASQLWDIAQARVCEVIVGILCGGMMMMILPSSSDATALLTALKNMHARLLEHASLLWQPETTDAIRAAHEGVIGQILTMNLLRIQAFWSHYRFRQQNARLNALLHQQLRMTSVISSLRRMLLNWPSPPGATREILEQLLTALASSQTDVYTVARIIAPLRPTNVADYRHVAFWQRLRYFCRLYLQSSQELHRLQSGVDDHTRLPRTSGLARHTDNAEAMWSGLRTFCTLMMIGAWSIASQWDAGANALTLAAISCVLYSAVAAPFKSLSLLMRTLVLLSLFSFVVKFGLMVQISDLWQFLLFLFPLLATMQLLKLQMPKFAALWGQLIVFMGSFIAVTNPPVYDFADFLNDNLAKIVGVALAWLAFAILRPGSDARKSRRHIRALRRDFVDQLSRHPTLSESEFESLTYHHVSQLSNSQDALARRWLLRWGVVLLNCSHVVWQLRDWESRSDPLSRVRDNCISLLRGVMSERGVQQKSLAATLEELQRICDSLARHHQPAARELAAIIWRLYCSLSQLEQAPPQGTLAS

SEQ ID NO: 11 - protein, 655 aa, synthetic construct
  REGION 1..655: note = aaeB
MGIFSIANQHIRFAVKLATAIVLALFVGFHFQLETPRWAVLTAAIVAAGTAFAAGGEPYSGAIRYRGFLRIIGTFIGCIAGLVIIIAMIRAPLLMILVCCIWAGFCTWISSLVRIENSYAWGLAGYTALIIVITIQPEPLLTPQFAVERCSEIVIGIVCAIMADLLFSPRSIKQEVDRELESLLVAQYQLMQLCIKHGDGEVVDKAWGDLVRRTTALQGMRSNLNMESSRWARANRRLKAINTLSLTLITQSCETYLIQNTRPELITDTFREFFDTPVETAQDVHKQLKRLRRVIAWTGERETPVTIYSWVAAATRYQLLKRGVISNTKINATEEEILQGEPEVKVESAERHHAMVNFWRTTLSCILGTLFWLWTGWTSGSGAMVMIAVVTSLAMRLPNPRMVAIDFIYGTLAALPLGLLYFLVIIPNTQQSMLLLCISLAVLGFFLGIEVQKRRLGSMGALASTINIIVLDNPMTFHFSQFLDSALGQIVGCVLAFTVILLVRDKSRDRTGRVLLNQFVSAAVSAMTTNVARRKENHLPALYQQLFLLMNKFPGDLPKFRLALTMIIAHQRLRDAPIPVNEDLSAFHRQMRRTADHVISARSDDKRRRYFGQLLEELEIYQEKLRIWQAPPQVTEPVNRLAGMLHKYQHALTDS

SEQ ID NO: 12 - protein, 352 aa, synthetic construct
  REGION 1..352: note = yeeA
VRADKSLSPFEIRVYRHYRIVHGTRVALAFLLTFLIIRLFTIPESTWPLVTMVVIMGPISFWGNVVPRAFERIGGTVLGSILGLIALQLELISLPLMLVWCAAAMFLCGWLALGKKPYQGLLIGVTLAIVVGSPTGEIDTALWRSGDVILGSLLAMLFTGIWPQRAFIHWRIQLAKSLTEYNRVYQSAFSPNLLERPRLESHLQKLLTDAVKMRGLIAPASKETRIPKSIYEGIQTINRNLVCMLELQINAYWATRPSHFVLLNAQKLRDTQHMMQQILLSLVHALYEGNPQPVFANTEKLNDAVEELRQLLNNHHDLKVVETPIYGYVWLNMETAHQLELLSNLICRALRK

SEQ ID NO: 13 - protein, 206 aa, synthetic construct
  REGION 1..206: note = rhtC
MLMLFLTVAMVHIVALMSPGPDFFFVSQTAVSRSRKEAMMGVLGITCGVMVWAGIALLGLHLIIEKMAWLHTLIMVGGGLYLCWMGYQMLRGALKKEAVSAPAPQVELAKSGRSFLKGLLTNLANPKAIIYFGSVFSLFVGDNVGTTARWGIFALIIVETLAWFTVVASLFALPQMRRGYQRLAKWIDGFAGALFAGFGIHLIISR

SEQ ID NO: 14 - protein, 394 aa, synthetic construct
  REGION 1..394: note = emrD
MKRQRNVNLLLMLVLLVAVGQMAQTIYIPAIADMARDLNVREGAVQSVMGAYLLTYGVSQLFYGPISDRVGRRPVILVGMSIFMLATLVAVTTSSLTVLIAASAMQGMGTGVGGVMARTLPRDLYERTQLRHANSLLNMGILVSPLLAPLIGGLLDTMWNWRACYLFLLVLCAGVTFSMARWMPETRPVDAPRTRLLTSYKTLFGNSGFNCYLLMLIGGLAGIAAFEACSGVLMGAVLGLSSMTVSILFILPIPAAFFGAWFAGRPNKRFSTLMWQSVICCLLAGLLMWIPDWFGVMNVWTLLVPAALFFFGAGMLFPLATSGAMEPFPFLAGTAGALVGGLQNIGSGVLASLSAMLPQTGQGSLGLLMTLMGLLIVLCWLPLATRMSHQGQPV

SEQ ID NO: 15 - DNA, 25 bp, synthetic construct
  misc_feature 1..25: note = yddG H1F
  source 1..25: mol_type = other DNA
caatgccgctactgttgttccagcc

SEQ ID NO: 16 - DNA, 25 bp, synthetic construct
  misc_feature 1..25: note = yddG H1R
  source 1..25: mol_type = other DNA
cagtggtgcgtttttctaccgctat

SEQ ID NO: 17 - DNA, 22 bp, synthetic construct
  misc_feature 1..22: note = yddG H2F
  source 1..22: mol_type = other DNA
aataactgccgggtctacggcc

SEQ ID NO: 18 - DNA, 33 bp, synthetic construct
  misc_feature 1..33: note = yddG H2R
  source 1..33: mol_type = other DNA
aacgtattttctaaacgaattttaaacggcgtc

SEQ ID NO: 19 - DNA, 26 bp, synthetic construct
  misc_feature 1..26: note = yddG CF
  source 1..26: mol_type = other DNA
cggaacagtatgtgcaggtgttacgg

SEQ ID NO: 20 - DNA, 26 bp, synthetic construct
  misc_feature 1..26: note = yddG CR
  source 1..26: mol_type = other DNA
aacaaaccagttacaaccaccgcaac

SEQ ID NO: 21 - DNA, 28 bp, synthetic construct
  misc_feature 1..28: note = yicL_F
  source 1..28: mol_type = other DNA
gcgagctcatgggttccaccagaaaggg

SEQ ID NO: 22 - DNA, 27 bp, synthetic construct
  misc_feature 1..27: note = yicL_R
  source 1..27: mol_type = other DNA
gctctagatcacttatgccgcgccgga

SEQ ID NO: 23 - DNA, 33 bp, synthetic construct
  misc_feature 1..33: note = ydiN_F
  source 1..33: mol_type = other DNA
gcgagctcatgtctcaaaataaggctttcagca

SEQ ID NO: 24 - DNA, 28 bp, synthetic construct
  misc_feature 1..28: note = ydiN_R
  source 1..28: mol_type = other DNA
gctctagaggccatcaacccaatcaatt

SEQ ID NO: 25 - DNA, 33 bp, synthetic construct
  misc_feature 1..33: note = ydhK_F
  source 1..33: mol_type = other DNA
gcgagctcatgaacgcatcgtcatggtccttgc

SEQ ID NO: 26 - DNA, 27 bp, synthetic construct
  misc_feature 1..27: note = ydhK_R
  source 1..27: mol_type = other DNA
gctctagatcacttatgccgcgccgga

SEQ ID NO: 27 - DNA, 29 bp, synthetic construct
  misc_feature 1..29: note = aaeB_F
  source 1..29: mol_type = other DNA
gcgagctcatgggtattttctccattgct

SEQ ID NO: 28 - DNA, 29 bp, synthetic construct
  misc_feature 1..29: note = aaeB_R
  source 1..29: mol_type = other DNA
gctctagattttgacttaactatcggtca

SEQ ID NO: 29 - DNA, 25 bp, synthetic construct
  misc_feature 1..25: note = yeeA_F
  source 1..25: mol_type = other DNA
gcgagctcgtgcgtgccgataagtc

SEQ ID NO: 30 - DNA, 26 bp, synthetic construct
  misc_feature 1..26: note = yeeA_R
  source 1..26: mol_type = other DNA
gctctagattatttgcgcaaggcccg

SEQ ID NO: 31 - DNA, 31 bp, synthetic construct
  misc_feature 1..31: note = rhtC_F
  source 1..31: mol_type = other DNA
gcgagctcatgttgatgttatttctcaccgt

SEQ ID NO: 32 - DNA, 28 bp, synthetic construct
  misc_feature 1..28: note = rhtC_R
  source 1..28: mol_type = other DNA
gctctagactggcatcaccgcgaaataa

SEQ ID NO: 33 - DNA, 27 bp, synthetic construct
  misc_feature 1..27: note = emrD_F
  source 1..27: mol_type = other DNA
gcgagctcatgaaaaggcaaagaaacg

SEQ ID NO: 34 - DNA, 27 bp, synthetic construct
  misc_feature 1..27: note = emrD_R
  source 1..27: mol_type = other DNA
gctctagacggtgacgtgcgcttaaac

SEQ ID NO: 35 - DNA, 24 bp, synthetic construct
  misc_feature 1..24: note = primer_F
  source 1..24: mol_type = other DNA
gcgccgacatcataacggttctgg

SEQ ID NO: 36 - DNA, 23 bp, synthetic construct
  misc_feature 1..23: note = primer_R
  source 1..23: mol_type = other DNA
cgcaacgttcaaatccgctcccg

SEQ ID NO: 37 - DNA, 2013 bp, synthetic construct
  misc_feature 1..2013: note = ydhK 1945G
  source 1..2013: mol_type = other DNA
atgaacgcatcgtcatggtccttgcgcaatttgccctggttcagggccacgctggcgcaatggcgttatgcgttacgcaataccattgccatgtgtctggcgctgacggttgcctattatttaaatctggatgaaccctattgggcgatgacctcggctgcagtggttagctttcccaccgttggcggtgttatcagcaaaagcctcggacgcatcgctggcagtttgctcggagccattgcggcactgcttcttgccgggcatacgctcaatgagccgtggttttttctattgagcatgtcggcgtggcttggcttttgtacctgggcctgtgcgcacttcacgaataacgtcgcgtatgcatttcaactggcgggctacacggctgccatcatcgcctttccgatggttaatattactgaggccagccagctgtgggatatcgctcaggcgcgcgtttgcgaggtaatagtcggtattttgtgcggcggcatgatgatgatgatcctgccgagcagttccgatgctactgcccttttaaccgcattgaaaaacatgcacgcccgattactggaacatgccagtttactctggcagcctgaaacaaccgatgccattcgtgcagcacatgaaggggtgattgggcagatactgaccatgaatttgctgcgtatccaggctttctggagccactatcgttttcgccagcaaaacgcgcgccttaatgcgctgctccaccagcaattacgtatgaccagtgtcatctccagcctgcgacgtatgttgctcaactggccctcaccgccaggtgccacacgagaaattctcgaacagttgctgacggcgctcgccagttcgcaaacagatgtttacaccgtcgcacgtattatcgccccgctacgcccgaccaacgtcgccgactatcggcacgtcgccttctggcagcgactacgttatttttgccgcctttatctgcaaagtagtcaggaattacatcgtctgcaaagcggtgtagatgatcataccagactcccacggacatccggcctggctcgtcataccgataacgccgaagctatgtggagcgggctgcgtacattttgtacgttgatgatgattggcgcatggagtattgcttcgcaatgggatgccggtgccaatgcattaacgctggcagcaattagctgcgtactctactccgccgtcgcagcaccgtttaagtcgttgtcacttctgatgcgcacgctggtgttactttcgctattcagctttgtggtcaaatttggtctgatggtccagattagcgatctgtggcaatttttactgtttctctttccactgctggcgacaatgcagcttcttaaattgcagatgccaaaatttgccgcattgtgggggcaactgattgtttttatgggttcttttatcgctgtcactaatcccccggtgtatgattttgctgattttcttaacgataatctggcaaaaatcgttggcgtcgcgttggcgtggttagcgttcgccattctgcgtccaggatcggatgctcgtaaaagccgccgccatattcgcgcgctgcgccgggattttgtcgatcagctaagccgccatccaacactgagtgaaagcgaatttgaatcgctcacttatcatcacgtcagtcagttgagtaacagccaggatgcgctggctcgccgttggttattacgctggggtgtagtgctgctgaactgttctcatgttgtctggcaattgcgcgactgggaatcgcgttccgatccgttatcgcgagtacgggataactgtatttcactgttgcggggagtgatgagtgagcgtggcgttcagcaaaaatcactggcggccacacttgaagaattacagcggatttgcgacagccttgcccgtcatcatcaacctgccgcccgtgagctggcggcaattgtctggcggctgtactgctcgctttcgcaacttgagcaagcaccaccgcaaggtacgctggcctcttaa

SEQ ID NO: 38 - protein, 670 aa, synthetic construct
  REGION 1..670: note = ydhK 649V
MNASSWSLRNLPWFRATLAQWRYALRNTIAMCLALTVAYYLNLDEPYWAMTSAAVVSFPTVGGVISKSLGRIAGSLLGAIAALLLAGHTLNEPWFFLLSMSAWLGFCTWACAHFTNNVAYAFQLAGYTAAIIAFPMVNITEASQLWDIAQARVCEVIVGILCGGMMMMILPSSSDATALLTALKNMHARLLEHASLLWQPETTDAIRAAHEGVIGQILTMNLLRIQAFWSHYRFRQQNARLNALLHQQLRMTSVISSLRRMLLNWPSPPGATREILEQLLTALASSQTDVYTVARIIAPLRPTNVADYRHVAFWQRLRYFCRLYLQSSQELHRLQSGVDDHTRLPRTSGLARHTDNAEAMWSGLRTFCTLMMIGAWSIASQWDAGANALTLAAISCVLYSAVAAPFKSLSLLMRTLVLLSLFSFVVKFGLMVQISDLWQFLLFLFPLLATMQLLKLQMPKFAALWGQLIVFMGSFIAVTNPPVYDFADFLNDNLAKIVGVALAWLAFAILRPGSDARKSRRHIRALRRDFVDQLSRHPTLSESEFESLTYHHVSQLSNSQDALARRWLLRWGVVLLNCSHVVWQLRDWESRSDPLSRVRDNCISLLRGVMSERGVQQKSLAATLEELQRICDSLARHHQPAARELAAIVWRLYCSLSQLEQAPPQGTLAS

SEQ ID NO: 39 - DNA, 1185 bp, synthetic construct
  misc_feature 1..1185: note = ermD 1071G
  source 1..1185: mol_type = other DNA
atgaaaaggcaaagaaacgtcaatttgttattgatgttggtattactcgtggccgtcggtcagatggcgcaaaccatttatattccagctattgccgatatggcgcgcgatctcaacgtccgtgaaggggcggtgcagagcgtaatgggcgcttatctgctgacttacggtgtctcacagctgttttatggcccgatttccgaccgcgtgggccgccgaccggtgatcctcgtcggaatgtccatttttatgctggcaacgctggtcgcggtcacgacctccagtttgacggtgttgattgccgccagcgcgatgcaggggatgggcaccggcgttggcggcgtaatggcgcgtactttaccgcgagatttatatgaacggacacagttgcgccatgctaacagcctgttaaacatggggattctcgtcagtccgttgctcgcaccgctaatcggcggtctgctggatacgatgtggaactggcgcgcctgttatctctttttgttggttctttgtgctggtgtgaccttcagtatggcccgctggatgccggaaacgcgtccggtcgatgcaccgcgcacgcgcctgcttaccagttataaaacgcttttcggtaacagcggttttaactgttatttgctgatgctgattggcggtctggccgggattgccgcctttgaagcctgctccggcgtgctgatgggcgcggtgttagggctgagcagtatgacggtcagtattttgtttattctgccgattccggcagcgttttttggcgcatggtttgccggacgtcccaataaacgcttctccacgttaatgtggcagtcggttatctgctgcctgctggctggcttgctgatgtggatccccgactggtttggcgtgatgaatgtctggacgctgctcgttcccgccgcgctgttctttttcggtgccgggatgctgtttccgctggcgaccagcggcgcgatggagccgttccccttcctggcgggcacggctggcgcgctggtcggcggtctgcaaaacattggttccggcgtgctggcgtcgctctctgcgatgttgccgcaaaccggtcagggcagcctggggttgttgatgaccttaatgggattgttgatcgtgctgtgctggctgccgctggcgacgcggatgtcgcatcaggggcagcccgtttaa